European Patent Specification EP 3 337 819 B1, published February 21, 2024. Title: PURIFICATION OF FKPA AND USES THEREOF FOR PRODUCING RECOMBINANT POLYPEPTIDES. Applicant: GENENTECH, INC. ET AL LADIWALA, Asif MCKAY, Patrick A. FONG, Chris B. Application Not Yet Assigned. The sequence listing filed with the application follows.

SEQUENCE LISTING (45 sequences)

SEQ ID NO: 1 - protein, 185 aa, Escherichia coli
AFADKSKLSDQEIEQTLQAFEARVKSSAQAKMEKDAADNEAKGKEYREKFAKEKGVKTSSTGLVYQVVEAGKGEAPKDSDTVVVNYKGTLIDGKEFDNSYTRGEPLSFRLDGVIPGWTEGLKNIKKGGKIKLVIPPELAYGKAGVPGIPPNSTLVFDVELLDVKPAPKADAKPEADAKAADSAKK

SEQ ID NO: 2 - protein, 270 aa, Escherichia coli
  MOD_RES (239)..(239): Any amino acid
MKSLFKVTLLATTMAVALHAPITFAAEAAKPATTADSKAAFKNDDQKSAYALGASLGRYMENSLKEQEKLGIKLDKDQLIAGVQDAFADKSKLSDQEIEQTLQAFEARVKSSAQAKMEKDAADNEAKGKEYREKFAKEKGVKTSSTGLVYQVVEAGKGEAPKDSDTVVVNYKGTLIDGKEFDNSYTRGEPLSFRLDGVIPGWTEGLKNIKKGGKIKLVIPPELAYGKAGVPGIPPNSTXVFDVELLDVKPAPKADAKPEADAKAADSAKK

SEQ ID NO: 3 - DNA, 813 bp, Escherichia coli
atgaaatcactgtttaaagtaacgctgctggcgaccacaatggccgttgccctgcatgcaccaatcacttttgctgctgaagctgcaaaacctgctacagctgctgacagcaaagcagcgttcaaaaatgacgatcagaaatcagcttatgcactgggtgcctcgctgggtcgttacatggaaaactctctaaaagaacaagaaaaactgggcatcaaactggataaagatcagctgatcgctggtgttcaggatgcatttgctgataagagcaaactctccgaccaagagatcgaacagactctacaagcattcgaagctcgcgtgaagtcttctgctcaggcgaagatggaaaaagacgcggctgataacgaagcaaaaggtaaagagtaccgcgagaaatttgccaaagagaaaggtgtgaaaacctcttcaactggtctggtttatcaggtagtagaagccggtaaaggcgaagcaccgaaagacagcgatactgttgtagtgaactacaaaggtacgctgatcgacggtaaagagttcgacaactcttacacccgtggtgaaccgctttctttccgtctggacggtgttatcccgggttggacagaaggtctgaagaacatcaagaaaggcggtaagatcaaactggttattccaccagaactggcttacggcaaagcgggtgttccggggatcccaccgaattctaccctggtgtttgacgtagagctgctggatgtgaaaccagcgccgaaggctgatgcaaagccggaagctgatgcgaaagccgcagattctgctaaaaaataa

SEQ ID NO: 4 - protein, 132 aa, Homo sapiens
MALLLTTVIALTCLGGFASPGPVPPSTALRELIEELVNITQNQKAPLCNGSMVWSINLTAGMYCAALESLINVSGCSAIEKTQRMLSGFCPHKVSAGQFSSLHVRDTKIEVAQFVKDLLLHLKKLFREGRFN

SEQ ID NO: 5 - protein, 114 aa, Homo sapiens
SPGPVPPSTALRELIEELVNITQNQKAPLCNGSMVWSINLTAGMYCAALESLINVSGCSAIEKTQRMLSGFCPHKVSAGQFSSLHVRDTKIEVAQFVKDLLLHLKKLFREGRFN

SEQ ID NO: 6 - protein, 155 aa, Homo sapiens
MTPGKTSLVSLLLLLSLEAIVKAGITIPRNPGCPNSEDKNFPRTVMVNLNIHNRNTNTNPKRSSDYYNRSTSPWNLHRNEDPERYPSVIWEAKCRHLGCINADGNVDYHMNSVPIQQEILVLRREPPHCPNSFRLEKILVSVGCTCVTPIVHHVA

SEQ ID NO: 7 - protein, 132 aa, Homo sapiens
GITIPRNPGCPNSEDKNFPRTVMVNLNIHNRNTNTNPKRSSDYYNRSTSPWNLHRNEDPERYPSVIWEAKCRHLGCINADGNVDYHMNSVPIQQEILVLRREPPHCPNSFRLEKILVSVGCTCVTPIVHHVA

SEQ ID NO: 8 - protein, 163 aa, Homo sapiens
MTVKTLHGPAMVKYLLLSILGLAFLSEAAARKIPKVGHTFFQKPESCPPVPGGSMKLDIGIINENQRVSMSRNIESRSTSPWNYTVTWDPNRYPSEVVQAQCRNLGCINAQGKEDISMNSVPIQQETLVVRRKHQGCSVSFQLEKVLVTVGCTCVTPVIHHVQ

SEQ ID NO: 9 - protein, 133 aa, Homo sapiens [sequence omitted]

SEQ ID NO: 10 - protein, 118 aa, Artificial Sequence
  synthetic construct
EVTLRESGPALVKPTQTLTLTCTVSGFSLSAYSVNWIRQPPGKALEWLAMIWGDGKIVYNSALKSRLTISKDTSKNQVVLTMTNMDPVDTATYYCAGDGYYPYAMDNWGQGSLVTVSS

SEQ ID NO: 11 - protein, 112 aa, Artificial Sequence
  synthetic construct
DIVLTQSPDSLSVSLGERATINCRASKSVDSYGNSFMHWYQQKPGQPPKLLIYLASNLESGVPDRFSGSGSGTDFTLTISSLQAEDVAVYYCQQNNEDPRTFGGGTKVEIKR

SEQ ID NO: 12 - protein, 5 aa, Artificial Sequence
  synthetic construct
AYSVN

SEQ ID NO: 13 - protein, 16 aa, Artificial Sequence
  synthetic construct
MIWGDGKIVYNSALKS

SEQ ID NO: 14 - protein, 10 aa, Artificial Sequence
  synthetic construct
DGYYPYAMDN

SEQ ID NO: 15 - protein, 15 aa, Artificial Sequence
  synthetic construct
RASKSVDSYGNSFMH

SEQ ID NO: 16 - protein, 7 aa, Artificial Sequence
  synthetic construct
LASNLES

SEQ ID NO: 17 - protein, 9 aa, Artificial Sequence
  synthetic construct
QQNNEDPRT

SEQ ID NO: 18 - protein, 444 aa, Artificial Sequence
  synthetic construct
EVTLRESGPALVKPTQTLTLTCTVSGFSLSAYSVNWIRQPPGKALEWLAMIWGDGKIVYNSALKSRLTISKDTSKNQVVLTMTNMDPVDTATYYCAGDGYYPYAMDNWGQGSLVTVSSASTKGPSVFPLAPCSRSTSESTAALGCLVKDYFPEPVTVSWNSGALTSGVHTFPAVLQSSGLYSLSSVVTVPSSSLGTKTYTCNVDHKPSNTKVDKRVESKYGPPCPPCPAPEFLGGPSVFLFPPKPKDTLMISRTPEVTCVVVDVSQEDPEVQFNWYVDGVEVHNAKTKPREEQFNSTYRVVSVLTVLHQDWLNGKEYKCKVSNKGLPSSIEKTISKAKGQPREPQVYTLPPSQEEMTKNQVSLWCLVKGFYPSDIAVEWESNGQPENNYKTTPPVLDSDGSFFLYSRLTVDKSRWQEGNVFSCSVMHEALHNHYTQKSLSLSLG

SEQ ID NO: 19 - protein, 445 aa, Artificial Sequence
  synthetic construct
EVTLRESGPALVKPTQTLTLTCTVSGFSLSAYSVNWIRQPPGKALEWLAMIWGDGKIVYNSALKSRLTISKDTSKNQVVLTMTNMDPVDTATYYCAGDGYYPYAMDNWGQGSLVTVSSASTKGPSVFPLAPCSRSTSESTAALGCLVKDYFPEPVTVSWNSGALTSGVHTFPAVLQSSGLYSLSSVVTVPSSSLGTKTYTCNVDHKPSNTKVDKRVESKYGPPCPPCPAPEFLGGPSVFLFPPKPKDTLMISRTPEVTCVVVDVSQEDPEVQFNWYVDGVEVHNAKTKPREEQFNSTYRVVSVLTVLHQDWLNGKEYKCKVSNKGLPSSIEKTISKAKGQPREPQVYTLPPSQEEMTKNQVSLWCLVKGFYPSDIAVEWESNGQPENNYKTTPPVLDSDGSFFLYSRLTVDKSRWQEGNVFSCSVMHEALHNHYTQKSLSLSLGK

SEQ ID NO: 20 - protein, 218 aa, Artificial Sequence
  synthetic construct
DIVLTQSPDSLSVSLGERATINCRASKSVDSYGNSFMHWYQQKPGQPPKLLIYLASNLESGVPDRFSGSGSGTDFTLTISSLQAEDVAVYYCQQNNEDPRTFGGGTKVEIKRTVAAPSVFIFPPSDEQLKSGTASVVCLLNNFYPREAKVQWKVDNALQSGNSQESVTEQDSKDSTYSLSSTLTLSKADYEKHKVYACEVTHQGLSSPVTKSFNRGEC

SEQ ID NO: 21 - protein, 123 aa, Artificial Sequence
  synthetic construct
EVQLVESGGGLVQPGRSLRLSCAASGFTFDDYAMHWVRQAPGKGLEWVSGINWSSGGIGYADSVKGRFTISRDNAKNSLYLQMNSLRAEDTALYYCARDIGGFGEFYWNFGLWGRGTLVTVSS

SEQ ID NO: 22 - protein, 108 aa, Artificial Sequence
  synthetic construct
EIVLTQSPATLSLSPGERATLSCRASQSVRSYLAWYQQKPGQAPRLLIYDASNRATGIPARFSGSGSGTDFTLTISSLEPEDFAVYYCQQRSNWPPATFGGGTKVEIK

SEQ ID NO: 23 - protein, 5 aa, Artificial Sequence
  synthetic construct
DYAMH

SEQ ID NO: 24 - protein, 17 aa, Artificial Sequence
  synthetic construct
GINWSSGGIGYADSVKG

SEQ ID NO: 25 - protein, 14 aa, Artificial Sequence
  synthetic construct
DIGGFGEFYWNFGL

SEQ ID NO: 26 - protein, 11 aa, Artificial Sequence
  synthetic construct
RASQSVRSYLA

SEQ ID NO: 27 - protein, 7 aa, Artificial Sequence
  synthetic construct
DASNRAT

SEQ ID NO: 28 - protein, 10 aa, Artificial Sequence
  synthetic construct
QQRSNWPPAT

SEQ ID NO: 29 - protein, 449 aa, Artificial Sequence
  synthetic construct
EVQLVESGGGLVQPGRSLRLSCAASGFTFDDYAMHWVRQAPGKGLEWVSGINWSSGGIGYADSVKGRFTISRDNAKNSLYLQMNSLRAEDTALYYCARDIGGFGEFYWNFGLWGRGTLVTVSSASTKGPSVFPLAPCSRSTSESTAALGCLVKDYFPEPVTVSWNSGALTSGVHTFPAVLQSSGLYSLSSVVTVPSSSLGTKTYTCNVDHKPSNTKVDKRVESKYGPPCPPCPAPEFLGGPSVFLFPPKPKDTLMISRTPEVTCVVVDVSQEDPEVQFNWYVDGVEVHNAKTKPREEQFNSTYRVVSVLTVLHQDWLNGKEYKCKVSNKGLPSSIEKTISKAKGQPREPQVYTLPPSQEEMTKNQVSLSCAVKGFYPSDIAVEWESNGQPENNYKTTPPVLDSDGSFFLVSRLTVDKSRWQEGNVFSCSVMHEALHNHYTQKSLSLSLG

SEQ ID NO: 30 - protein, 450 aa, Artificial Sequence
  synthetic construct
EVQLVESGGGLVQPGRSLRLSCAASGFTFDDYAMHWVRQAPGKGLEWVSGINWSSGGIGYADSVKGRFTISRDNAKNSLYLQMNSLRAEDTALYYCARDIGGFGEFYWNFGLWGRGTLVTVSSASTKGPSVFPLAPCSRSTSESTAALGCLVKDYFPEPVTVSWNSGALTSGVHTFPAVLQSSGLYSLSSVVTVPSSSLGTKTYTCNVDHKPSNTKVDKRVESKYGPPCPPCPAPEFLGGPSVFLFPPKPKDTLMISRTPEVTCVVVDVSQEDPEVQFNWYVDGVEVHNAKTKPREEQFNSTYRVVSVLTVLHQDWLNGKEYKCKVSNKGLPSSIEKTISKAKGQPREPQVYTLPPSQEEMTKNQVSLSCAVKGFYPSDIAVEWESNGQPENNYKTTPPVLDSDGSFFLVSRLTVDKSRWQEGNVFSCSVMHEALHNHYTQKSLSLSLGK

SEQ ID NO: 31 - protein, 215 aa, Artificial Sequence
  synthetic construct
EIVLTQSPATLSLSPGERATLSCRASQSVRSYLAWYQQKPGQAPRLLIYDASNRATGIPARFSGSGSGTDFTLTISSLEPEDFAVYYCQQRSNWPPATFGGGTKVEIKRTVAAPSVFIFPPSDEQLKSGTASVVCLLNNFYPREAKVQWKVDNALQSGNSQESVTEQDSKDSTYSLSSTLTLSKADYEKHKVYACEVTHQGLSSPVTKSFNRGEC

SEQ ID NO: 32 - DNA, 354 bp, Artificial Sequence
  synthetic construct
gaagttaccctgcgcgagagcggcccagccctggtgaagccaacccagaccctgaccctgacctgcaccgtcagcggcttcagcctgagcgcctacagcgtgaactggatccgccagccaccaggcaaggccctggagtggctggccatgatctggggcgacggcaagatcgtgtacaacagcgccctgaagagccgcctgaccatcagcaaggacaccagcaagaaccaggtggtgctgaccatgaccaacatggacccagtggacaccgccacctactactgcgccggcgacggctactacccatacgccatggacaactggggccagggcagcctggtgaccgtgagcagc

SEQ ID NO: 33 - DNA, 333 bp, Artificial Sequence
  synthetic construct
gatatcgtgctgacccagagcccagacagcctgtctgtgagcctgggcgagcgcgccaccatcaactgccgcgccagcaaaagcgtggacagctacggcaacagcttcatgcactggtatcagcagaagccaggccagccacccaagctgctgatctacctggccagcaacctggagagcggcgtgccagaccgcttcagcggcagcggcagcggcaccgacttcaccctgaccatcagctctctgcaggccgaggatgtggccgtgtactactgccagcagaacaacgaggacccacgcaccttcggtggcggtaccaaggtggagatcaaa

SEQ ID NO: 34 - DNA, 1332 bp, Artificial Sequence
  synthetic construct
gaagttaccctgcgcgagagcggcccagccctggtgaagccaacccagaccctgaccctgacctgcaccgtcagcggcttcagcctgagcgcctacagcgtgaactggatccgccagccaccaggcaaggccctggagtggctggccatgatctggggcgacggcaagatcgtgtacaacagcgccctgaagagccgcctgaccatcagcaaggacaccagcaagaaccaggtggtgctgaccatgaccaacatggacccagtggacaccgccacctactactgcgccggcgacggctactacccatacgccatggacaactggggccagggcagcctggtgaccgtgagcagcgcttccaccaagggcccatcggtcttccccctggcaccctgctcccgcagtacttctgagtccacagcggccctgggctgcctggtcaaggactacttccccgaaccggtgacggtgtcgtggaactcaggcgccctgaccagcggcgtgcacaccttcccggctgtcctacagtcctcaggactctactccctcagcagcgtggtgactgtgccctctagcagcttgggcaccaagacctacacgtgcaacgtggatcacaagcccagcaacaccaaggtggacaaacgcgttgagtccaaatatggtcccccatgcccaccatgcccagcacctgagttcctggggggaccatcagtcttcctgttccccccaaaacccaaggacactctcatgatctcccggacccctgaggtcacgtgcgtggtggtggacgtgagccaggaagaccccgaggtccagttcaactggtacgtggatggcgtggaggtgcataatgccaagacaaagccgcgggaggagcagttcaacagcacgtaccgtgtggtcagcgtcctcaccgtcctgcaccaggactggctgaacggcaaggagtacaagtgcaaggtctccaacaaaggcctcccgtcctccatcgagaaaaccatctccaaagccaaagggcagccccgagagccacaggtgtacaccctgcccccatcccaggaggagatgaccaagaaccaggtcagcctgtggtgcctggtcaaaggcttctaccccagcgacatcgccgtggagtgggagagcaatgggcagccggagaacaactacaagaccacgcctcccgtgctggactccgacggctccttcttcctctacagcaggctaaccgtggacaagagcaggtggcaggaggggaatgtcttctcatgctccgtgatgcatgaggctctgcacaaccactacacacagaagagcctctccctgtctctgggt

SEQ ID NO: 35 - DNA, 1338 bp, Artificial Sequence
  synthetic construct
gaagttaccctgcgcgagagcggcccagccctggtgaagccaacccagaccctgaccctgacctgcaccgtcagcggcttcagcctgagcgcctacagcgtgaactggatccgccagccaccaggcaaggccctggagtggctggccatgatctggggcgacggcaagatcgtgtacaacagcgccctgaagagccgcctgaccatcagcaaggacaccagcaagaaccaggtggtgctgaccatgaccaacatggacccagtggacaccgccacctactactgcgccggcgacggctactacccatacgccatggacaactggggccagggcagcctggtgaccgtgagcagcgcttccaccaagggcccatcggtcttccccctggcaccctgctcccgcagtacttctgagtccacagcggccctgggctgcctggtcaaggactacttccccgaaccggtgacggtgtcgtggaactcaggcgccctgaccagcggcgtgcacaccttcccggctgtcctacagtcctcaggactctactccctcagcagcgtggtgactgtgccctctagcagcttgggcaccaagacctacacgtgcaacgtggatcacaagcccagcaacaccaaggtggacaaacgcgttgagtccaaatatggtcccccatgcccaccatgcccagcacctgagttcctggggggaccatcagtcttcctgttccccccaaaacccaaggacactctcatgatctcccggacccctgaggtcacgtgcgtggtggtggacgtgagccaggaagaccccgaggtccagttcaactggtacgtggatggcgtggaggtgcataatgccaagacaaagccgcgggaggagcagttcaacagcacgtaccgtgtggtcagcgtcctcaccgtcctgcaccaggactggctgaacggcaaggagtacaagtgcaaggtctccaacaaaggcctcccgtcctccatcgagaaaaccatctccaaagccaaagggcagccccgagagccacaggtgtacaccctgcccccatcccaggaggagatgaccaagaaccaggtcagcctgtggtgcctggtcaaaggcttctaccccagcgacatcgccgtggagtgggagagcaatgggcagccggagaacaactacaagaccacgcctcccgtgctggactccgacggctccttcttcctctacagcaggctaaccgtggacaagagcaggtggcaggaggggaatgtcttctcatgctccgtgatgcatgaggctctgcacaaccactacacacagaagagcctctccctgtctctgggtaaataa

SEQ ID NO: 36 - DNA, 657 bp, Artificial Sequence
  synthetic construct
gatatcgtgctgacccagagcccagacagcctgtctgtgagcctgggcgagcgcgccaccatcaactgccgcgccagcaaaagcgtggacagctacggcaacagcttcatgcactggtatcagcagaagccaggccagccacccaagctgctgatctacctggccagcaacctggagagcggcgtgccagaccgcttcagcggcagcggcagcggcaccgacttcaccctgaccatcagctctctgcaggccgaggatgtggccgtgtactactgccagcagaacaacgaggacccacgcaccttcggtggcggtaccaaggtggagatcaaacgaactgtggctgcaccatctgtcttcatcttcccgccatctgatgagcagttgaaatctggaactgcttctgttgtgtgcctgctgaataacttctatccccgtgaggccaaagtacagtggaaggtggataacgccctccaatcgggtaactcccaggagagtgtcacagagcaggacagcaaggacagcacctacagcctcagcagcaccctgacgctgagcaaagcagactacgagaaacacaaagtctacgcctgcgaagtcacccatcagggcctgagctcgcccgtcacaaagagcttcaacaggggagagtgttaa

SEQ ID NO: 37 - DNA, 369 bp, Artificial Sequence
  synthetic construct
gaagtgcagctggtggagtctgggggaggcttggtacagcctggcaggtccctgagactctcctgtgcagcctctggattcacctttgatgattatgccatgcactgggtccggcaagctccagggaagggcctggagtgggtctcaggtattaattggagcagtggtggcataggctatgcggactctgtgaagggccgattcaccatctccagagacaacgccaagaactccctgtatctgcaaatgaacagtctgagagctgaggacacggccttgtattactgtgcaagagatatcggggggttcggggagttttactggaacttcggtctctggggccgtggcaccctggtcactgtctcctca

SEQ ID NO: 38 - DNA, 324 bp, Artificial Sequence
  synthetic construct
gaaattgtgttgacacagtctccagccaccctgtctttgtctccaggggaaagagccaccctctcctgcagggccagtcagagtgttagaagctacttagcctggtaccaacagaaacctggccaggctcccaggctcctcatctatgatgcatccaacagggccactggcatcccagccaggttcagtggcagtgggtctgggacagacttcactctcaccatcagcagcctagagcctgaagattttgcagtttattactgtcagcagcgtagcaactggcctccggccactttcggcggagggaccaaggtggagatcaaa

SEQ ID NO: 39 - DNA, 1347 bp, Artificial Sequence
  synthetic construct
gaagtgcagctggtggagtctgggggaggcttggtacagcctggcaggtccctgagactctcctgtgcagcctctggattcacctttgatgattatgccatgcactgggtccggcaagctccagggaagggcctggagtgggtctcaggtattaattggagcagtggtggcataggctatgcggactctgtgaagggccgattcaccatctccagagacaacgccaagaactccctgtatctgcaaatgaacagtctgagagctgaggacacggccttgtattactgtgcaagagatatcggggggttcggggagttttactggaacttcggtctctggggccgtggcaccctggtcactgtctcctcagcctccaccaagggcccatcggtcttccccctggcaccctgctcccgcagtacttctgagtccacagcggccctgggctgcctggtcaaggactacttccccgaaccggtgacggtgtcgtggaactcaggcgccctgaccagcggcgtgcacaccttcccggctgtcctacagtcctcaggactctactccctcagcagcgtggtgactgtgccctctagcagcttgggcaccaagacctacacgtgcaacgtggatcacaagcccagcaacaccaaggtggacaaacgcgttgagtccaaatatggtcccccatgcccaccatgcccagcacctgagttcctggggggaccatcagtcttcctgttccccccaaaacccaaggacactctcatgatctcccggacccctgaggtcacgtgcgtggtggtggacgtgagccaggaagaccccgaggtccagttcaactggtacgtggatggcgtggaggtgcataatgccaagacaaagccgcgggaggagcagttcaacagcacgtaccgtgtggtcagcgtcctcaccgtcctgcaccaggactggctgaacggcaaggagtacaagtgcaaggtctccaacaaaggcctcccgtcctccatcgagaaaaccatctccaaagccaaagggcagccccgagagccacaggtgtacaccctgcccccatcccaggaggagatgaccaagaaccaggtcagcctgagctgcgctgtcaaaggcttctaccccagcgacatcgccgtggagtgggagagcaatgggcagccggagaacaactacaagaccacgcctcccgtgctggactccgacggctccttcttcctcgttagcaggctaaccgtggacaagagcaggtggcaggaggggaatgtcttctcatgctccgtgatgcatgaggctctgcacaaccactacacacagaagagcctctccctgtctctgggt

SEQ ID NO: 40 - DNA, 1353 bp, Artificial Sequence
  synthetic construct
gaagtgcagctggtggagtctgggggaggcttggtacagcctggcaggtccctgagactctcctgtgcagcctctggattcacctttgatgattatgccatgcactgggtccggcaagctccagggaagggcctggagtgggtctcaggtattaattggagcagtggtggcataggctatgcggactctgtgaagggccgattcaccatctccagagacaacgccaagaactccctgtatctgcaaatgaacagtctgagagctgaggacacggccttgtattactgtgcaagagatatcggggggttcggggagttttactggaacttcggtctctggggccgtggcaccctggtcactgtctcctcagcctccaccaagggcccatcggtcttccccctggcaccctgctcccgcagtacttctgagtccacagcggccctgggctgcctggtcaaggactacttccccgaaccggtgacggtgtcgtggaactcaggcgccctgaccagcggcgtgcacaccttcccggctgtcctacagtcctcaggactctactccctcagcagcgtggtgactgtgccctctagcagcttgggcaccaagacctacacgtgcaacgtggatcacaagcccagcaacaccaaggtggacaaacgcgttgagtccaaatatggtcccccatgcccaccatgcccagcacctgagttcctggggggaccatcagtcttcctgttccccccaaaacccaaggacactctcatgatctcccggacccctgaggtcacgtgcgtggtggtggacgtgagccaggaagaccccgaggtccagttcaactggtacgtggatggcgtggaggtgcataatgccaagacaaagccgcgggaggagcagttcaacagcacgtaccgtgtggtcagcgtcctcaccgtcctgcaccaggactggctgaacggcaaggagtacaagtgcaaggtctccaacaaaggcctcccgtcctccatcgagaaaaccatctccaaagccaaagggcagccccgagagccacaggtgtacaccctgcccccatcccaggaggagatgaccaagaaccaggtcagcctgagctgcgctgtcaaaggcttctaccccagcgacatcgccgtggagtgggagagcaatgggcagccggagaacaactacaagaccacgcctcccgtgctggactccgacggctccttcttcctcgttagcaggctaaccgtggacaagagcaggtggcaggaggggaatgtcttctcatgctccgtgatgcatgaggctctgcacaaccactacacacagaagagcctctccctgtctctgggtaaataa

SEQ ID NO: 41 - DNA, 648 bp, Artificial Sequence
  synthetic construct
gaaattgtgttgacacagtctccagccaccctgtctttgtctccaggggaaagagccaccctctcctgcagggccagtcagagtgttagaagctacttagcctggtaccaacagaaacctggccaggctcccaggctcctcatctatgatgcatccaacagggccactggcatcccagccaggttcagtggcagtgggtctgggacagacttcactctcaccatcagcagcctagagcctgaagattttgcagtttattactgtcagcagcgtagcaactggcctccggccactttcggcggagggaccaaggtggagatcaaacgaactgtggctgcaccatctgtcttcatcttcccgccatctgatgagcagttgaaatctggaactgcttctgttgtgtgcctgctgaataacttctatccccgtgaggccaaagtacagtggaaggtggataacgccctccaatcgggtaactcccaggagagtgtcacagagcaggacagcaaggacagcacctacagcctcagcagcaccctgacgctgagcaaagcagactacgagaaacacaaagtctacgcctgcgaagtcacccatcagggcctgagctcgcccgtcacaaagagcttcaacaggggagagtgttaa

SEQ ID NO: 42 - DNA, 1347 bp, Artificial Sequence
  synthetic construct
gaagttcagctggttgaaagcggtggtggtctggttcagcctggtcgtagcctgcgtctgagctgtgcagcaagcggttttacctttgatgattatgccatgcattgggttcgtcaggcaccgggtaaaggtctggaatgggttagcggtattaattggagcagcggtggtattggttatgcagatagcgttaaaggtcgttttaccattagccgtgataatgccaaaaatagcctgtacctgcagatgaatagtctgcgtgcagaagataccgcactgtattattgtgcacgtgatattggtggttttggcgaattctattggaattttggtctgtggggtcgtggcaccctggttaccgttagcagcgcctccaccaagggcccatcggtcttccccctggcaccctgctcccgcagtacttctgagtccacagcggccctgggctgcctggtcaaggactacttccccgaaccggtgacggtgtcgtggaactcaggcgccctgaccagcggcgtgcacaccttcccggctgtcctacagtcctcaggactctactccctcagcagcgtggtgactgtgccctctagcagcttgggcaccaagacctacacgtgcaacgtggatcacaagcccagcaacaccaaggtggacaaacgcgttgagtccaaatatggtcccccatgcccaccatgcccagcacctgagttcctggggggaccatcagtcttcctgttccccccaaaacccaaggacactctcatgatctcccggacccctgaggtcacgtgcgtggtggtggacgtgagccaggaagaccccgaggtccagttcaactggtacgtggatggcgtggaggtgcataatgccaagacaaagccgcgggaggagcagttcaacagcacgtaccgtgtggtcagcgtcctcaccgtcctgcaccaggactggctgaacggcaaggagtacaagtgcaaggtctccaacaaaggcctcccgtcctccatcgagaaaaccatctccaaagccaaagggcagccccgagagccacaggtgtacaccctgcccccatcccaggaggagatgaccaagaaccaggtcagcctgagctgcgctgtcaaaggcttctaccccagcgacatcgccgtggagtgggagagcaatgggcagccggagaacaactacaagaccacgcctcccgtgctggactccgacggctccttcttcctcgttagcaggctaaccgtggacaagagcaggtggcaggaggggaatgtcttctcatgctccgtgatgcatgaggctctgcacaaccactacacacagaagagcctctccctgtctctgggt

SEQ ID NO: 43 - DNA, 1353 bp, Artificial Sequence
  synthetic construct
gaagttcagctggttgaaagcggtggtggtctggttcagcctggtcgtagcctgcgtctgagctgtgcagcaagcggttttacctttgatgattatgccatgcattgggttcgtcaggcaccgggtaaaggtctggaatgggttagcggtattaattggagcagcggtggtattggttatgcagatagcgttaaaggtcgttttaccattagccgtgataatgccaaaaatagcctgtacctgcagatgaatagtctgcgtgcagaagataccgcactgtattattgtgcacgtgatattggtggttttggcgaattctattggaattttggtctgtggggtcgtggcaccctggttaccgttagcagcgcctccaccaagggcccatcggtcttccccctggcaccctgctcccgcagtacttctgagtccacagcggccctgggctgcctggtcaaggactacttccccgaaccggtgacggtgtcgtggaactcaggcgccctgaccagcggcgtgcacaccttcccggctgtcctacagtcctcaggactctactccctcagcagcgtggtgactgtgccctctagcagcttgggcaccaagacctacacgtgcaacgtggatcacaagcccagcaacaccaaggtggacaaacgcgttgagtccaaatatggtcccccatgcccaccatgcccagcacctgagttcctggggggaccatcagtcttcctgttccccccaaaacccaaggacactctcatgatctcccggacccctgaggtcacgtgcgtggtggtggacgtgagccaggaagaccccgaggtccagttcaactggtacgtggatggcgtggaggtgcataatgccaagacaaagccgcgggaggagcagttcaacagcacgtaccgtgtggtcagcgtcctcaccgtcctgcaccaggactggctgaacggcaaggagtacaagtgcaaggtctccaacaaaggcctcccgtcctccatcgagaaaaccatctccaaagccaaagggcagccccgagagccacaggtgtacaccctgcccccatcccaggaggagatgaccaagaaccaggtcagcctgagctgcgctgtcaaaggcttctaccccagcgacatcgccgtggagtgggagagcaatgggcagccggagaacaactacaagaccacgcctcccgtgctggactccgacggctccttcttcctcgttagcaggctaaccgtggacaagagcaggtggcaggaggggaatgtcttctcatgctccgtgatgcatgaggctctgcacaaccactacacacagaagagcctctccctgtctctgggtaaataa

SEQ ID NO: 44 - DNA, 648 bp, Artificial Sequence
  synthetic construct
gaaattgttctgacccagagtccggcaaccctgagcctgagtccgggtgaacgtgccaccctgagctgtcgtgcaagccagagcgttcgtagctatctggcatggtatcagcagaaaccgggtcaggcaccgcgtctgctgatttatgatgcaagcaatcgtgcaaccggtattccggcacgttttagcggtagcggtagtggcaccgattttaccctgaccattagcagcctggaaccggaagattttgcagtgtattattgtcagcagcgtagcaattggccaccggcaacctttggtggtggcaccaaagttgaaattaaacgaactgtggctgcaccatctgtcttcatcttcccgccatctgatgagcagttgaaatctggaactgcttctgttgtgtgcctgctgaataacttctatccccgtgaggccaaagtacagtggaaggtggataacgccctccaatcgggtaactcccaggagagtgtcacagagcaggacagcaaggacagcacctacagcctcagcagcaccctgacgctgagcaaagcagactacgagaaacacaaagtctacgcctgcgaagtcacccatcagggcctgagctcgcccgtcacaaagagcttcaacaggggagagtgttaa

SEQ ID NO: 45 - protein, 11 aa, Escherichia coli
SAYALGASLGR